European Patent Application EP 4 144 758 A1, published March 8, 2023. Title: SINGLE VARIABLE DOMAIN ANTIBODY TARGETING HUMAN PROGRAMMED DEATH LIGAND 1 (PD-L1) AND DERIVATIVE THEREOF. Applicant: Mabwell (Shanghai) Bioscience Co Ltd. The sequence listing filed with the application follows.

SEQUENCE LISTING (45 sequences)

SEQ ID NO: 1 - protein, 120 aa, VHH-F2
QVQLQESGGGSVQTGGSLRLACAVSRDSDDGASCMGWFRQAPGKGREGVAIIFNAGERTDYGDSVKGRFTISQDNAKNTLFLQMNSLKPEDSAMYYCATVWCGSWVARSFGQGTQVTVSS

SEQ ID NO: 2 - DNA, 360 bp, VHH-F2
caggtgcagctgcaggagtctggaggaggctcggtgcagactggagggtctctgagactcgcctgtgcagtctctagagacagtgacgacggtgccagctgtatggggtggttccgccaggctccagggaaggggcgcgagggggtcgcaatcatttttaatgctggtgaacgtaccgactatggcgactccgtgaagggccgattcaccatctcccaagacaacgccaagaacacgctgtttctacaaatgaacagcctgaaacctgaggacagtgccatgtactattgtgcgacagtttggtgtggttcttgggtcgcgcgttctttcggccaggggacccaggtcaccgtctcctca

SEQ ID NO: 3 - protein, 353 aa, chF2-C region
QVQLQESGGGSVQTGGSLRLACAVSRDSDDGASCMGWFRQAPGKGREGVAIIFNAGERTDYGDSVKGRFTISQDNAKNTLFLQMNSLKPEDSAMYYCATVWCGSWVARSFGQGTQVTVSSASEPKSSDKTHTCPPCPAPELLGGPSVFLFPPKPKDTLMISRTPEVTCVVVDVSHEDPEVKFNWYVDGVEVHNAKTKPREEQYNSTYRVVSVLTVLHQDWLNGKEYKCKVSNKALPAPIEKTISKAKGQPREPQVYTLPPSRDELTKNQVSLTCLVKGFYPSDIAVEWESNGQPENNYKTTPPVLDSDGSFFLYSKLTVDKSRWQQGNVFSCSVMHEALHNHYTQKSLSLSPG

SEQ ID NO: 4 - DNA, 1059 bp, chF2-C region
caggtgcagctgcaggagtctggaggaggctcggtgcagactggagggtctctgagactcgcctgtgcagtctctagagacagtgacgacggtgccagctgtatggggtggttccgccaggctccagggaaggggcgcgagggggtcgcaatcatttttaatgctggtgaacgtaccgactatggcgactccgtgaagggccgattcaccatctcccaagacaacgccaagaacacgctgtttctacaaatgaacagcctgaaacctgaggacagtgccatgtactattgtgcgacagtttggtgtggttcttgggtcgcgcgttctttcggccaggggacccaggtcaccgtctcctcagctagcgagcccaaatctagcgacaaaactcacacatgcccaccgtgcccagcacctgaactcctggggggaccgtcagtcttcctcttccccccaaaacccaaggacaccctcatgatctcccggacccctgaggtcacatgcgtggtggtggacgtgagccacgaagaccctgaggtcaagttcaactggtacgtggacggcgtggaggtgcataatgccaagacaaagccgcgggaggagcagtacaacagcacgtaccgtgtggtcagcgtcctcaccgtcctgcaccaggactggctgaatggcaaggagtacaagtgcaaggtctccaacaaagccctcccagcccccatcgagaaaaccatctccaaagccaaagggcagccccgagaaccacaggtgtacaccctgcctccatctcgggatgagctgaccaagaaccaggtcagcctgacctgcctggtcaaaggcttctatcccagcgacatcgccgtggagtgggagagcaatgggcagccggagaacaactacaagaccacgcctcccgtgctggactccgacggctccttcttcctctatagcaagctcaccgtggacaagagcaggtggcagcaggggaacgtcttctcatgctccgtgatgcatgaggctctgcacaaccactacacgcagaagagcctctccctgtccccgggt

SEQ ID NO: 5 - protein, 128 aa, KN035
QVQLVESGGGLVQPGGSLRLSCAASGKMSSRRCMAWFRQAPGKERERVAKLLTTSGSTYLADSVKGRFTISRDNSKNTVYLQMNSLRAEDTAVYYCAADSFEDPTCTLVTSSGAFQYWGQGTLVTVSS

SEQ ID NO: 6 - DNA, 384 bp, KN035
caggtgcagctggtggagtctggaggaggcctggtgcagcctggaggctccctgaggctgtcctgcgctgcctctggcaagatgtcctccagacggtgcatggcctggttccgacaggctcctggcaaggagcgagagcgggtggccaagctgctgaccacctccggctccacctacctggccgactccgtgaagggacggttcaccatctccagggacaactccaagaacaccgtgtacctgcagatgaactccctgcgagctgaggacaccgccgtgtactactgcgctgcagactccttcgaggaccccacctgcaccctggtgacctcctctggagccttccagtactggggacagggcaccctggtgaccgtgtcctcc

SEQ ID NO: 7 - protein, 120 aa, hzF2
EVQLVESGGGLVQPGGSLRLSCAASRDSDDGASCMGWFRQAPGKGLEGVAIIFNAGERTDYGDSVKGRFTISRDNAKNTLYLQMNSLRAEDTAVYYCATVWCGSWVARSWGQGTLVTVSS

SEQ ID NO: 8 - DNA, 360 bp, hzF2
gaggtgcagctggtggagtctggaggtggcctggtgcagcctggaggctccctgaggctgtcctgcgctgcctctcgggactccgacgacggagcctcctgcatgggctggttcaggcaggctcctggcaagggcctggagggagtggccatcatcttcaacgctggcgagcggaccgactacggcgactccgtgaagggacggttcaccatctccagggacaacgccaagaacaccctgtacctgcagatgaactccctgagagccgaggacacagccgtgtactactgcgctaccgtgtggtgtggctcctgggtggctcggtcctggggacagggcaccctggtgaccgtgtcctcc

SEQ ID NO: 9 - protein, 353 aa, hzF2-C region
EVQLVESGGGLVQPGGSLRLSCAASRDSDDGASCMGWFRQAPGKGLEGVAIIFNAGERTDYGDSVKGRFTISRDNAKNTLYLQMNSLRAEDTAVYYCATVWCGSWVARSWGQGTLVTVSSASEPKSSDKTHTCPPCPAPELLGGPSVFLFPPKPKDTLMISRTPEVTCVVVDVSHEDPEVKFNWYVDGVEVHNAKTKPREEQYNSTYRVVSVLTVLHQDWLNGKEYKCKVSNKALPAPIEKTISKAKGQPREPQVYTLPPSRDELTKNQVSLTCLVKGFYPSDIAVEWESNGQPENNYKTTPPVLDSDGSFFLYSKLTVDKSRWQQGNVFSCSVMHEALHNHYTQKSLSLSPG

SEQ ID NO: 10 - DNA, 1059 bp, hzF2-C region
gaggtgcagctggtggagtctggaggtggcctggtgcagcctggaggctccctgaggctgtcctgcgctgcctctcgggactccgacgacggagcctcctgcatgggctggttcaggcaggctcctggcaagggcctggagggagtggccatcatcttcaacgctggcgagcggaccgactacggcgactccgtgaagggacggttcaccatctccagggacaacgccaagaacaccctgtacctgcagatgaactccctgagagccgaggacacagccgtgtactactgcgctaccgtgtggtgtggctcctgggtggctcggtcctggggacagggcaccctggtgaccgtgtcctccgctagcgagcccaaatctagcgacaaaactcacacatgcccaccgtgcccagcacctgaactcctggggggaccgtcagtcttcctcttccccccaaaacccaaggacaccctcatgatctcccggacccctgaggtcacatgcgtggtggtggacgtgagccacgaagaccctgaggtcaagttcaactggtacgtggacggcgtggaggtgcataatgccaagacaaagccgcgggaggagcagtacaacagcacgtaccgtgtggtcagcgtcctcaccgtcctgcaccaggactggctgaatggcaaggagtacaagtgcaaggtctccaacaaagccctcccagcccccatcgagaaaaccatctccaaagccaaagggcagccccgagaaccacaggtgtacaccctgcctccatctcgggatgagctgaccaagaaccaggtcagcctgacctgcctggtcaaaggcttctatcccagcgacatcgccgtggagtgggagagcaatgggcagccggagaacaactacaagaccacgcctcccgtgctggactccgacggctccttcttcctctatagcaagctcaccgtggacaagagcaggtggcagcaggggaacgtcttctcatgctccgtgatgcatgaggctctgcacaaccactacacgcagaagagcctctccctgtccccgggt

SEQ ID NO: 11 - protein, 120 aa, hzF2-m1
EVQLVESGGGLVQPGGSLRLSCAASRDSDDGASSMGWFRQAPGKGLEGVAIIFNAGERTDYGDSVKGRFTISRDNAKNTLYLQMNSLRAEDTAVYYCATVWSGSWVARSWGQGTLVTVSS

SEQ ID NO: 12 - protein, 120 aa, hzF2-m2
EVQLVESGGGLVQPGGSLRLSCAASGDSDDGASCMGWFRQAPGKGLEGVAIIFNAGERTDYGDSVKGRFTISRDNAKNTLYLQMNSLRAEDTAVYYCATVWCGSWVARSWGQGTLVTVSS

SEQ ID NO: 13 - protein, 120 aa, hzF2-m3
EVQLVESGGGLVQPGGSLRLSCAASRDSSSGASCMGWFRQAPGKGLEGVAIIFNAGERTDYGDSVKGRFTISRDNAKNTLYLQMNSLRAEDTAVYYCATVWCGSWVARSWGQGTLVTVSS

SEQ ID NO: 14 - protein, 120 aa, hzF2-m4
EVQLVESGGGLVQPGGSLRLSCAASRDSNDGASCMGWFRQAPGKGLEGVAIIFNAGERTDYGDSVKGRFTISRDNAKNTLYLQMNSLRAEDTAVYYCATVWCGSWVARSWGQGTLVTVSS

SEQ ID NO: 15 - protein, 120 aa, hzF2-m5
EVQLVESGGGLVQPGGSLRLSCAASRDSDDAASCMGWFRQAPGKGLEGVAIIFNAGERTDYGDSVKGRFTISRDNAKNTLYLQMNSLRAEDTAVYYCATVWCGSWVARSWGQGTLVTVSS

SEQ ID NO: 16 - protein, 120 aa, hzF2-m6
EVQLVESGGGLVQPGGSLRLSCAASRDSDEGASCMGWFRQAPGKGLEGVAIIFNAGERTDYGDSVKGRFTISRDNAKNTLYLQMNSLRAEDTAVYYCATVWCGSWVARSWGQGTLVTVSS

SEQ ID NO: 17 - protein, 120 aa, hzF2-m7
EVQLVESGGGLVQPGGSLRLSCAASRDSDDSASCMGWFRQAPGKGLEGVAIIFNAGERTDYGDSVKGRFTISRDNAKNTLYLQMNSLRAEDTAVYYCATVWCGSWVARSWGQGTLVTVSS

SEQ ID NO: 18 - protein, 120 aa, hzF2-m8
EVQLVESGGGLVQPGGSLRLSCAASRDSDDGASCMGWFRQAPGKEREGVAIIFNVGERTDYGDSVKGRFTISRDNAKNTLYLQMNSLRAEDTAVYYCATVWCGSWVARSWGQGTLVTVSS

SEQ ID NO: 19 - protein, 120 aa, hzF2-m9
EVQLVESGGGLVQPGGSLRLSCAASRDSDEGASCMGWFRQAPGKEREGVAIIFNAGERTDYGDSVKGRFTISRDNAKNTLYLQMNSLRAEDTAVYYCATVWCGSWVARSWGQGTLVTVSS

SEQ ID NO: 20 - protein, 120 aa, hzF2-m10
EVQLVESGGGLVQPGGSLRLSCAASRDSDDGASCMGWFRQAPGKEREGVAIIFNAGERTDYGDSVKGRFTISRDNAKNTLYLQMNSLRAEDTAVYYCATVYCGSWVARSWGQGTLVTVSS

SEQ ID NO: 21 - protein, 120 aa, hzF2-m11
EVQLVESGGGLVQPGGSLRLSCAASRDSDDGASCMGWFRQAPGKEREGVAIIFNAGERTDYGDSVKGRFTISRDNAKNTLYLQMNSLRAEDTAVYYCATVYCGSYVARSWGQGTLVTVSS

SEQ ID NO: 22 - protein, 120 aa, hzF2-m12
EVQLVESGGGLVQPGGSLRLSCAASRDSDEGASCMGWFRQAPGKEREGVAIIFNVGERTDYGDSVKGRFTISRDNAKNTLYLQMNSLRAEDTAVYYCATVWCGSWVARSWGQGTLVTVSS

SEQ ID NO: 23 - protein, 120 aa, hzF2-m13
EVQLVESGGGLVQPGGSLRLSCAASRDSDDGASCMGWFRQAPGKEREGVAIIFNAGERTDYGDSVKGRFTISRDNAKNTLYLQMNSLRAEDTAVYYCATVFCGSFVARSWGQGTLVTVSS

SEQ ID NO: 24 - protein, 120 aa, hzF2-m14
EVQLVESGGGLVQPGGSLRLSCAASRDSDEGASCMGWFRQAPGKEREGVAIIFNVGERTDYGDSVKGRFTISRDNAKNTLYLQMNSLRAEDTAVYYCATVYCGSYVARSWGQGTLVTVSS

SEQ ID NO: 25 - protein, 120 aa, hzF2-m15
EVQLVESGGGLVQPGGSLRLSCAASRDSDEGASCMGWFRQAPGKEREGVAIIFNVGERTDYGDSVKGRFTISRDNAKNTLYLQMNSLRAEDTAVYYCATVFCGSYVARSWGQGTLVTVSS

SEQ ID NO: 26 - protein, 120 aa, hzF2-m16
EVQLVESGGGLVQPGGSLRLSCAASRDSDEGASCMGWFRQAPGKEREGVAIIFNVGERTDYGDSVKGRFTISRDNAKNTLYLQMNSLRAEDTAVYYCATVFCGSFVARSWGQGTLVTVSS

SEQ ID NO: 27 - DNA, 360 bp, hzF2-m1
gaggtgcagctggtggagtctggaggtggcctggtgcagcctggaggctccctgaggctgtcctgcgctgcctctcgggactccgacgacggagcctccagcatgggctggttcaggcaggctcctggcaagggcctggagggagtggccatcatcttcaacgctggcgagcggaccgactacggcgactccgtgaagggacggttcaccatctccagggacaacgccaagaacaccctgtacctgcagatgaactccctgagagccgaggacacagccgtgtactactgcgctaccgtgtggtccggctcctgggtggctcggtcctggggacagggcaccctggtgaccgtgtcctcc

SEQ ID NO: 28 - DNA, 360 bp, hzF2-m2
gaggtgcagctggtggagtctggaggtggcctggtgcagcctggaggctccctgaggctgtcctgcgctgcctctggagactccgacgacggagcctcctgcatgggctggttcaggcaggctcctggcaagggcctggagggagtggccatcatcttcaacgctggcgagcggaccgactacggcgactccgtgaagggacggttcaccatctccagggacaacgccaagaacaccctgtacctgcagatgaactccctgagagccgaggacacagccgtgtactactgcgctaccgtgtggtgtggctcctgggtggctcggtcctggggacagggcaccctggtgaccgtgtcctcc

SEQ ID NO: 29 - DNA, 360 bp, hzF2-m3
gaggtgcagctggtggagtctggaggtggcctggtgcagcctggaggctccctgaggctgtcctgcgctgcctctcgggactccagcagcggagcctcctgcatgggctggttcaggcaggctcctggcaagggcctggagggagtggccatcatcttcaacgctggcgagcggaccgactacggcgactccgtgaagggacggttcaccatctccagggacaacgccaagaacaccctgtacctgcagatgaactccctgagagccgaggacacagccgtgtactactgcgctaccgtgtggtgtggctcctgggtggctcggtcctggggacagggcaccctggtgaccgtgtcctcc

SEQ ID NO: 30 - DNA, 360 bp, hzF2-m4
gaggtgcagctggtggagtctggaggtggcctggtgcagcctggaggctccctgaggctgtcctgcgctgcctctcgggactccaacgacggagcctcctgcatgggctggttcaggcaggctcctggcaagggcctggagggagtggccatcatcttcaacgctggcgagcggaccgactacggcgactccgtgaagggacggttcaccatctccagggacaacgccaagaacaccctgtacctgcagatgaactccctgagagccgaggacacagccgtgtactactgcgctaccgtgtggtgtggctcctgggtggctcggtcctggggacagggcaccctggtgaccgtgtcctcc

SEQ ID NO: 31 - DNA, 360 bp, hzF2-m5
gaggtgcagctggtggagtctggaggtggcctggtgcagcctggaggctccctgaggctgtcctgcgctgcctctcgggactccgacgacgctgcctcctgcatgggctggttcaggcaggctcctggcaagggcctggagggagtggccatcatcttcaacgctggcgagcggaccgactacggcgactccgtgaagggacggttcaccatctccagggacaacgccaagaacaccctgtacctgcagatgaactccctgagagccgaggacacagccgtgtactactgcgctaccgtgtggtgtggctcctgggtggctcggtcctggggacagggcaccctggtgaccgtgtcctcc

SEQ ID NO: 32 - DNA, 360 bp, hzF2-m6
gaggtgcagctggtggagtctggaggtggcctggtgcagcctggaggctccctgaggctgtcctgcgctgcctctcgggactccgacgagggagcctcctgcatgggctggttcaggcaggctcctggcaagggcctggagggagtggccatcatcttcaacgctggcgagcggaccgactacggcgactccgtgaagggacggttcaccatctccagggacaacgccaagaacaccctgtacctgcagatgaactccctgagagccgaggacacagccgtgtactactgcgctaccgtgtggtgtggctcctgggtggctcggtcctggggacagggcaccctggtgaccgtgtcctcc

SEQ ID NO: 33 - DNA, 360 bp, hzF2-m7
gaggtgcagctggtggagtctggaggtggcctggtgcagcctggaggctccctgaggctgtcctgcgctgcctctcgggactccgacgactctgcctcctgcatgggctggttcaggcaggctcctggcaagggcctggagggagtggccatcatcttcaacgctggcgagcggaccgactacggcgactccgtgaagggacggttcaccatctccagggacaacgccaagaacaccctgtacctgcagatgaactccctgagagccgaggacacagccgtgtactactgcgctaccgtgtggtgtggctcctgggtggctcggtcctggggacagggcaccctggtgaccgtgtcctcc

SEQ ID NO: 34 - DNA, 360 bp, hzF2-m8
gaggtgcagctggtggagtctggaggtggcctggtgcagcctggaggctccctgaggctgtcctgcgctgcctctcgggactccgacgacggagcctcctgcatgggctggttcaggcaggctcctggcaaggagagagagggagtggccatcatcttcaacgtgggcgagcggaccgactacggcgactccgtgaagggacggttcaccatctccagggacaacgccaagaacaccctgtacctgcagatgaactccctgagagccgaggacacagccgtgtactactgcgctaccgtgtggtgtggctcctgggtggctcggtcctggggacagggcaccctggtgaccgtgtcctcc

SEQ ID NO: 35 - DNA, 360 bp, hzF2-m9
gaggtgcagctggtggagtctggaggtggcctggtgcagcctggaggctccctgaggctgtcctgcgctgcctctcgggactccgacgagggagcctcctgcatgggctggttcaggcaggctcctggcaaggagagagagggagtggccatcatcttcaacgctggcgagcggaccgactacggcgactccgtgaagggacggttcaccatctccagggacaacgccaagaacaccctgtacctgcagatgaactccctgagagccgaggacacagccgtgtactactgcgctaccgtgtggtgtggctcctgggtggctcggtcctggggacagggcaccctggtgaccgtgtcctcc

SEQ ID NO: 36 - DNA, 360 bp, hzF2-m10
gaggtgcagctggtggagtctggaggtggcctggtgcagcctggaggctccctgaggctgtcctgcgctgcctctcgggactccgacgacggagcctcctgcatgggctggttcaggcaggctcctggcaaggagagagagggagtggccatcatcttcaacgctggcgagcggaccgactacggcgactccgtgaagggacggttcaccatctccagggacaacgccaagaacaccctgtacctgcagatgaactccctgagagccgaggacacagccgtgtactactgcgctaccgtgtactgtggctcctgggtggctcggtcctggggacagggcaccctggtgaccgtgtcctcc

SEQ ID NO: 37 - DNA, 360 bp, hzF2-m11
gaggtgcagctggtggagtctggaggtggcctggtgcagcctggaggctccctgaggctgtcctgcgctgcctctcgggactccgacgacggagcctcctgcatgggctggttcaggcaggctcctggcaaggagagagagggagtggccatcatcttcaacgctggcgagcggaccgactacggcgactccgtgaagggacggttcaccatctccagggacaacgccaagaacaccctgtacctgcagatgaactccctgagagccgaggacacagccgtgtactactgcgctaccgtgtactgtggctcctacgtggctcggtcctggggacagggcaccctggtgaccgtgtcctcc

SEQ ID NO: 38 - DNA, 360 bp, hzF2-m12
gaggtgcagctggtggagtctggaggtggcctggtgcagcctggaggctccctgaggctgtcctgcgctgcctctcgggactccgacgagggagcctcctgcatgggctggttcaggcaggctcctggcaaggagagagagggagtggccatcatcttcaacgtgggcgagcggaccgactacggcgactccgtgaagggacggttcaccatctccagggacaacgccaagaacaccctgtacctgcagatgaactccctgagagccgaggacacagccgtgtactactgcgctaccgtgtggtgtggctcctgggtggctcggtcctggggacagggcaccctggtgaccgtgtcctcc

SEQ ID NO: 39 - DNA, 360 bp, hzF2-m13
gaggtgcagctggtggagtctggaggtggcctggtgcagcctggaggctccctgaggctgtcctgcgctgcctctcgggactccgacgacggagcctcctgcatgggctggttcaggcaggctcctggcaaggagagagagggagtggccatcatcttcaacgctggcgagcggaccgactacggcgactccgtgaagggacggttcaccatctccagggacaacgccaagaacaccctgtacctgcagatgaactccctgagagccgaggacacagccgtgtactactgcgctaccgtgttctgtggctccttcgtggctcggtcctggggacagggcaccctggtgaccgtgtcctcc

SEQ ID NO: 40 - DNA, 360 bp, hzF2-m14
gaggtgcagctggtggagtctggaggtggcctggtgcagcctggaggctccctgaggctgtcctgcgctgcctctcgggactccgacgagggagcctcctgcatgggctggttcaggcaggctcctggcaaggagagagagggagtggccatcatcttcaacgtgggcgagcggaccgactacggcgactccgtgaagggacggttcaccatctccagggacaacgccaagaacaccctgtacctgcagatgaactccctgagagccgaggacacagccgtgtactactgcgctaccgtgtactgtggctcctacgtggctcggtcctggggacagggcaccctggtgaccgtgtcctcc

SEQ ID NO: 41 - DNA, 360 bp, hzF2-m15
gaggtgcagctggtggagtctggaggtggcctggtgcagcctggaggctccctgaggctgtcctgcgctgcctctcgggactccgacgagggagcctcctgcatgggctggttcaggcaggctcctggcaaggagagagagggagtggccatcatcttcaacgtgggcgagcggaccgactacggcgactccgtgaagggacggttcaccatctccagggacaacgccaagaacaccctgtacctgcagatgaactccctgagagccgaggacacagccgtgtactactgcgctaccgtgttctgtggctcctacgtggctcggtcctggggacagggcaccctggtgaccgtgtcctcc

SEQ ID NO: 42 - DNA, 360 bp, hzF2-m16
gaggtgcagctggtggagtctggaggtggcctggtgcagcctggaggctccctgaggctgtcctgcgctgcctctcgggactccgacgagggagcctcctgcatgggctggttcaggcaggctcctggcaaggagagagagggagtggccatcatcttcaacgtgggcgagcggaccgactacggcgactccgtgaagggacggttcaccatctccagggacaacgccaagaacaccctgtacctgcagatgaactccctgagagccgaggacacagccgtgtactactgcgctaccgtgttctgtggctccttcgtggctcggtcctggggacagggcaccctggtgaccgtgtcctcc

SEQ ID NO: 43 - protein, 11 aa, VHH-F2 CDR1
RDSDDGASCMG

SEQ ID NO: 44 - protein, 17 aa, VHH-F2 CDR2
IIFNAGERTDYGDSVKG

SEQ ID NO: 45 - protein, 10 aa, VHH-F2 CDR3
VWCGSWVARS